European Patent Specification EP 3 611 272 B9, published October 4, 2023. Title: DETECTION REAGENT, DETECTION KIT AND DETECTION METHOD FOR ITGA4 GENE METHYLATION. Applicant: CREATIVE BIOSCIENCES (GUANGZHOU) CO., LTD. The sequence listing filed with the application follows.

SEQUENCE LISTING (24 sequences)

SEQ ID NO: 1 - DNA, 33 bp, Artificial sequence
  capturing sequence
tgcttctccgggtacgggccgctgggtggggtc

SEQ ID NO: 2 - DNA, 23 bp, Artificial sequence
  Upstream primer of ITGA4
tcggagaagtagcgcgagtattc

SEQ ID NO: 3 - DNA, 20 bp, Artificial sequence
  Downstream primer of ITGA4
aaatcgacccaccgcgaacg

SEQ ID NO: 4 - DNA, 19 bp, Artificial sequence
  Upstream primer of Set 1
acgcgagttttgcgtagtc

SEQ ID NO: 5 - DNA, 19 bp, Artificial sequence
  Downstream primer of Set 1
tccgaatacgaaccgctaa

SEQ ID NO: 6 - DNA, 23 bp, Artificial sequence
  Probe of Set 1
acggagttcggttttgcgttttc

SEQ ID NO: 7 - DNA, 20 bp, Artificial sequence
  Upstream primer of Set 2
gttttcgtattacgttcggg

SEQ ID NO: 8 - DNA, 20 bp, Artificial sequence
  Downstream primer of Set 2
tcgaaccgacctaaaatacc

SEQ ID NO: 9 - DNA, 22 bp, Artificial sequence
  Probe of Set 2
aatcgggagtggggtcgggcga

SEQ ID NO: 10 - DNA, 20 bp, Artificial sequence
  Upstream primer of Set 3
tatcgagagcgtatggtttg

SEQ ID NO: 11 - DNA, 20 bp, Artificial sequence
  Downstream primer of Set 3
ccacgttataaaaacgaccg

SEQ ID NO: 12 - DNA, 23 bp, artificial sequence
  Probe of Set 3
agggtcgtcgttcgggagacggt

SEQ ID NO: 13 - DNA, 20 bp, Artificial sequence
  Upstream primer of Set 4
agagttatttcgcgttttgc

SEQ ID NO: 14 - DNA, 20 bp, Artificial sequence
  Downstream primer of Set 4
atcccgaacgtaatacgaaa

SEQ ID NO: 15 - DNA, 24 bp, Artificial sequence
  Probe of Set 4
tgggaggttcgggttaggacgcga

SEQ ID NO: 16 - DNA, 20 bp, Artificial sequence
  Upstream primer of Set 5
tgcgttttcgtattacgttc

SEQ ID NO: 17 - DNA, 20 bp, Artificial sequence
  Downstream primer of Set 5
ccaaccgaaaacttcgaata

SEQ ID NO: 18 - DNA, 27 bp, Artificial sequence
  Probe of Set 5
gcggttcgtattcggagaagtagcgcg

SEQ ID NO: 19 - DNA, 20 bp, Artificial sequence
  Upstream primer of Set 6
gcggttcgtattcggagaag

SEQ ID NO: 20 - DNA, 20 bp, Artificial sequence
  Downstream primer of Set 6
tctaccgccaaccgaaaact

SEQ ID NO: 21 - DNA, 13 bp, Artificial sequence
  Probe of Set 6
agcgcgagtattc

SEQ ID NO: 22 - DNA, 17 bp, Artificial sequence
  Upstream primer of Set 7
tgcggaggcgtagggtc

SEQ ID NO: 23 - DNA, 19 bp, Artificial sequence
  Downstream primer of Set 7
caaccgaaattccccaacg

SEQ ID NO: 24 - DNA, 26 bp, Artificial sequence
  Probe of Set 7
cctacaaccgcgcgtaaacaaaaacg